European Patent Application EP 4 410 968 A1, published August 7, 2024. Title: MODIFIED ENZYME AND METHOD OF PRODUCING IMIDAZOLE DIPEPTIDE USING SAME. Applicant: Ajinomoto Co., Inc. The sequence listing filed with the application follows.

SEQUENCE LISTING (26 sequences)

SEQ ID NO: 1 - protein, 383 aa, Rhodotorula minuta
MERKRIRELLPNLRFGQFPTGPKNSLTDVPGVLVSTKSVIKPADLPHHHEVNTGVTTILPRKEWFKQGCYASYFRFNGSGEMTGSHWIDESGLLNSPVIITNSFGVGACYNGVYEYAKKHHKDEKGICDWFLTPVIAETFDGWLSDIGAMAVQSSDVVEGIENASSDAVPEGCTGGGTGMITMGFKAGTGNASRVIDSVKIDSKGEKQQVKYTLAALVQSNFGGARFLTVNGVPVGRILEDEAMAAKKAGPMDGPEGSIIVVIATDAPLIPIQLQRLAKRATVGVARTGGWGSNYSGDIFLAFSTAHEIPRENTQNWTPSVPQPQEVLDTESINALFEAAFEAVEEAIYNAICMATDTKGPDGREVKAIDLEKLKEIVTRHAY

SEQ ID NO: 2 - DNA, 250 bp, Escherichia coli
  source 1..250: mol_type = other DNA
gaataataaaagcgtgttatactctttccctgcaatgggttccgtagcagggaaagagaccccgttgtctcttcccggtatttcatctctatgtcacattttgtgcgtaatttattcacaagcttgcattgaacttgtggataaaatcacggtctgataaaacagtgaatgataacctcgttgctcttaagctctggcacagttgttgctaccactgaagcgccagaagatatcgattgagaggatttga

SEQ ID NO: 3 - DNA, 32 bp, synthetic construct
  misc_feature 1..32: note = Primer
  source 1..32: mol_type = other DNA
atggctgccgcgcggcaccaggccgctgctgt

SEQ ID NO: 4 - DNA, 30 bp, synthetic construct
  misc_feature 1..30: note = Primer
  source 1..30: mol_type = other DNA
ctcgagcaccaccaccaccaccactgagat

SEQ ID NO: 5 - DNA, 53 bp, synthetic construct
  misc_feature 1..53: note = Primer
  source 1..53: mol_type = other DNA
ccgcgcggcagccatatggaacgtaaacgcattcgcgaactgctcccgaattt

SEQ ID NO: 6 - DNA, 53 bp, synthetic construct
  misc_feature 1..53: note = Primer
  source 1..53: mol_type = other DNA
gtggtggtgctcgagttaataggcatggcgggtaacaatttctttgagtttct

SEQ ID NO: 7 - DNA, 27 bp, synthetic construct
  misc_feature 1..27: note = Primer
  source 1..27: mol_type = other DNA
gttaaatttgacagcaaaggcgagaaa

SEQ ID NO: 8 - DNA, 27 bp, synthetic construct
  misc_feature 1..27: note = Primer
  source 1..27: mol_type = other DNA
gctgtcaaatttaacggaatcgatcac

SEQ ID NO: 9 - DNA, 27 bp, synthetic construct
  misc_feature 1..27: note = Primer
  source 1..27: mol_type = other DNA
aagaaatttggcccaatggatgggccg

SEQ ID NO: 10 - DNA, 27 bp, synthetic construct
  misc_feature 1..27: note = Primer
  source 1..27: mol_type = other DNA
tgggccaaatttcttcgccgccattgc

SEQ ID NO: 11 - DNA, 27 bp, synthetic construct
  misc_feature 1..27: note = Primer
  source 1..27: mol_type = other DNA
aagaaattgggcccaatggatgggccg

SEQ ID NO: 12 - DNA, 27 bp, synthetic construct
  misc_feature 1..27: note = Primer
  source 1..27: mol_type = other DNA
tgggcccaatttcttcgccgccattgc

SEQ ID NO: 13 - DNA, 27 bp, synthetic construct
  misc_feature 1..27: note = Primer
  source 1..27: mol_type = other DNA
tggggttttaactactctggcgacatc

SEQ ID NO: 14 - DNA, 27 bp, synthetic construct
  misc_feature 1..27: note = Primer
  source 1..27: mol_type = other DNA
gtagttaaaaccccagccacctgtacg

SEQ ID NO: 15 - DNA, 27 bp, synthetic construct
  misc_feature 1..27: note = Primer
  source 1..27: mol_type = other DNA
ggaatggttaccatgggcttcaaagct

SEQ ID NO: 16 - DNA, 27 bp, synthetic construct
  misc_feature 1..27: note = Primer
  source 1..27: mol_type = other DNA
catggtaaccattccggtacctccgcc

SEQ ID NO: 17 - DNA, 27 bp, synthetic construct
  misc_feature 1..27: note = Primer
  source 1..27: mol_type = other DNA
aaaggagtttgcgactggttcctgact

SEQ ID NO: 18 - DNA, 27 bp, synthetic construct
  misc_feature 1..27: note = Primer
  source 1..27: mol_type = other DNA
gtcgcaaactcctttctcatccttgtg

SEQ ID NO: 19 - DNA, 27 bp, synthetic construct
  misc_feature 1..27: note = Primer
  source 1..27: mol_type = other DNA
ggttcgcattactctggcgacatcttt

SEQ ID NO: 20 - DNA, 27 bp, synthetic construct
  misc_feature 1..27: note = Primer
  source 1..27: mol_type = other DNA
agagtaatgcgaaccccagccacctgt

SEQ ID NO: 21 - DNA, 27 bp, synthetic construct
  misc_feature 1..27: note = Primer
  source 1..27: mol_type = other DNA
tctggcgatatgaccggctcccattgg

SEQ ID NO: 22 - DNA, 27 bp, synthetic construct
  misc_feature 1..27: note = Primer
  source 1..27: mol_type = other DNA
ggtcatatcgccagagccgttgaaccg

SEQ ID NO: 23 - DNA, 27 bp, synthetic construct
  misc_feature 1..27: note = Primer
  source 1..27: mol_type = other DNA
gaagcattggcggcgaagaaagcaggc

SEQ ID NO: 24 - DNA, 27 bp, synthetic construct
  misc_feature 1..27: note = Primer
  source 1..27: mol_type = other DNA
cgccgccaatgcttcatcttcgagaat

SEQ ID NO: 25 - DNA, 27 bp, synthetic construct
  misc_feature 1..27: note = Primer
  source 1..27: mol_type = other DNA
aaaggattgtgcgactggttcctgact

SEQ ID NO: 26 - DNA, 27 bp, synthetic construct
  misc_feature 1..27: note = Primer
  source 1..27: mol_type = other DNA
gtcgcacaatcctttctcatccttgtg